European Patent Application EP 4 810 625 A1, published September 23, 2026. Title: METHODS AND COMPOSITIONS FOR COMBINATORIAL INDEXING OF BEAD BASED NUCLEIC ACIDS. Applicant: Illumina, Inc. Application EP, filed May 15, 2026. The sequence listing filed with the application follows.

SEQUENCE LISTING (16 sequences)

SEQ ID NO: 1 - DNA, 20 bp, synthetic construct
  misc_feature 1..20: note = Artificial oligonucleotides
  source 1..20: mol_type = other DNA
aatgatacggcgaccaccga

SEQ ID NO: 2 - DNA, 24 bp, synthetic construct
  misc_feature 1..24: note = Artificial oligonucleotides
  source 1..24: mol_type = other DNA
caagcagaagacggcatacgagat

SEQ ID NO: 3 - DNA, 16 bp, synthetic construct
  misc_feature 1..16: note = Artificial oligonucleotides
  source 1..16: mol_type = other DNA
atgctctagacaagtc

SEQ ID NO: 4 - DNA, 12 bp, synthetic construct
  misc_feature 1..12: note = Artificial oligonucleotides
  source 1..12: mol_type = other DNA
tgctctacaagc

SEQ ID NO: 5 - DNA, 12 bp, synthetic construct
  misc_feature 1..12: note = Artificial oligonucleotides
  source 1..12: mol_type = other DNA
gctctaacaagc

SEQ ID NO: 6 - DNA, 12 bp, synthetic construct
  misc_feature 1..12: note = Artificial oligonucleotides
  source 1..12: mol_type = other DNA
gctctaacaagc

SEQ ID NO: 7 - DNA, 14 bp, synthetic construct
  misc_feature 1..14: note = Artificial oligonucleotides
  source 1..14: mol_type = other DNA
gacttgtccggtgg

SEQ ID NO: 8 - DNA, 14 bp, synthetic construct
  misc_feature 1..14: note = Artificial oligonucleotides
  source 1..14: mol_type = other DNA
ctgaacaggccacc

SEQ ID NO: 9 - DNA, 12 bp, synthetic construct
  misc_feature 1..12: note = Artificial oligonucleotides
  source 1..12: mol_type = other DNA
ctgaacaggcca

SEQ ID NO: 10 - DNA, 12 bp, synthetic construct
  misc_feature 1..12: note = Artificial oligonucleotides
  source 1..12: mol_type = other DNA
gaacaggccacc

SEQ ID NO: 11 - DNA, 15 bp, synthetic construct
  misc_feature 1..15: note = Artificial oligonucleotides
  misc_feature 15: note = N is inosine
  source 1..15: mol_type = other DNA
ctgaacaggccaccn

SEQ ID NO: 12 - DNA, 16 bp, synthetic construct
  misc_feature 1..16: note = CTGAACAGGCCACCNN
  misc_feature 15: note = N is Inosine
  source 1..16: mol_type = other DNA
  misc_feature 16: note = N is Inosine
ctgaacaggccaccnn

SEQ ID NO: 13 - DNA, 14 bp, synthetic construct
  misc_feature 1..14: note = Artificial oligonucleotides
  misc_feature 13: note = N is inosine
  source 1..14: mol_type = other DNA
  misc_feature 14: note = N is inosine
ctgaacaggccann

SEQ ID NO: 14 - DNA, 16 bp, synthetic construct
  misc_feature 1..16: note = Artificial oligonucleotides
  misc_feature 13: note = N is inosine
  source 1..16: mol_type = other DNA
  misc_feature 14: note = N is inosine
  misc_feature 15: note = N is inosine
  misc_feature 16: note = N is inosine
ctgaacaggccannnn

SEQ ID NO: 15 - DNA, 16 bp, synthetic construct
  misc_feature 1..16: note = Artificial oligonucleotide
  source 1..16: mol_type = other DNA
gacttgtctagagcat

SEQ ID NO: 16 - DNA, 16 bp, synthetic construct
  misc_feature 1..16: note = Artificial oligonucleotide
  source 1..16: mol_type = other DNA
ctgaacagatctcgta